European Patent Specification EP 2 647 706 B1, published May 17, 2023. Title: ANTIGEN-BINDING MOLECULES THAT REPEATEDLY BIND TO MULTIPLE ANTIGEN MOLECULES. Applicant: CHUGAI SEIYAKU KABUSHIKI KAISHA. The sequence listing filed with the application follows.

SEQUENCE LISTING (113 sequences)

SEQ ID NO: 1 - protein, 449 aa, Artificial Sequence
  an artificially synthesized sequence
QVQLVQSGAEVKKPGASVKVSCKASGYTFTSYYMHWVRQAPGQGLEWMGIINPSGGSTSYAQKFQGRVTMTRDTSTSTVYMELSSLRSEDTAVYYCARDDPGGGEYYFDYWGQGTLVTVSSASTKGPSVFPLAPSSKSTSGGTAALGCLVKDYFPEPVTVSWNSGALTSGVHTFPAVLQSSGLYSLSSVVTVPSSSLGTQTYICNVNHKPSNTKVDKKVEPKSCDKTHTCPPCPAPELLGGPSVFLFPPKPKDTLMISRTPEVTCVVVDVSHEDPEVKFNWYVDGVEVHNAKTKPREEQYNSTYRVVSVLTVLHQDWLNGKEYKCKVSNKALPAPIEKTISKAKGQPREPQVYTLPPSRDELTKNQVSLTCLVKGFYPSDIAVEWESNGQPENNYKTTPPVLDSDGSFFLYSKLTVDKSRWQQGNVFSCSVMHEALHNHYTQKSLSLSP

SEQ ID NO: 2 - protein, 216 aa, Artificial Sequence
  an artificially synthesized sequence
QSVLTQPPSVSGAPGQRVTISCTGSRSNMGAGYDVHWYQLLPGAAPKLLISHNTHRPSGVPDRFSGSKSGASASLAITGLQAEDEADYYCQSHDSSLSAVVFGGGTKLTVLSQPKAAPSVTLFPPSSEELQANKATLVCLISDFYPGAVTVAWKADSSPVKAGVETTTPSKQSNNKYAASSYLSLTPEQWKSHRSYSCQVTHEGSTVEKTVAPTEC

SEQ ID NO: 3 - protein, 453 aa, Artificial Sequence
  an artificially synthesized sequence
QVQLVQSGAEVKKPGSSVKVSCKASGGTFSSYAISWVRQAPGQGLEWMGGIIPIFGTANYAQKFQGRVTITADESTSTAYMELSSLRSEDTAVYYCARERDYYDSSGYYDAFDIWGQGTMVTVSSASTKGPSVFPLAPSSKSTSGGTAALGCLVKDYFPEPVTVSWNSGALTSGVHTFPAVLQSSGLYSLSSVVTVPSSSLGTQTYICNVNHKPSNTKVDKKVEPKSCDKTHTCPPCPAPELLGGPSVFLFPPKPKDTLMISRTPEVTCVVVDVSHEDPEVKFNWYVDGVEVHNAKTKPREEQYNSTYRVVSVLTVLHQDWLNGKEYKCKVSNKALPAPIEKTISKAKGQPREPQVYTLPPSRDELTKNQVSLTCLVKGFYPSDIAVEWESNGQPENNYKTTPPVLDSDGSFFLYSKLTVDKSRWQQGNVFSCSVMHEALHNHYTQKSLSLSP

SEQ ID NO: 4 - protein, 214 aa, Artificial Sequence
  an artificially synthesized sequence
ETTVTQSPSFLSASVGDRVTITCITTTDIDDDMNWFQQEPGKAPKLLISEGNILRPGVPSRFSSSGYGTDFTLTISKLQPEDFATYYCLQSDNLPFTFGQGTKLEIKRTVAAPSVFIFPPSDEQLKSGTASVVCLLNNFYPREAKVQWKVDNALQSGNSQESVTEQDSKDSTYSLSSTLTLSKADYEKHKVYACEVTHQGLSSPVTKSFNRGEC

SEQ ID NO: 5 - protein, 447 aa, Artificial Sequence
  an artificially synthesized sequence
QVQLQESGPGLVKPSETLSLTCAVSGYSISDDQAWSWVRQPPGEGLEWIGYISYSGITNYNPSLKGRVTISRDTSKNQFSLKLSSVTAADTAAYYCARSLARTTAMDYWGEGTLVTVSSASTKGPSVFPLAPSSKSTSGGTAALGCLVKDYFPEPVTVSWNSGALTSGVHTFPAVLQSSGLYSLSSVVTVPSSSLGTQTYICNVNHKPSNTKVDKKVEPKSCDKTHTCPPCPAPELLGGPSVFLFPPKPKDTLMISRTPEVTCVVVDVSHEDPEVKFNWYVDGVEVHNAKTKPREEQYNSTYRVVSVLTVLHQDWLNGKEYKCKVSNKALPAPIEKTISKAKGQPREPQVYTLPPSRDELTKNQVSLTCLVKGFYPSDIAVEWESNGQPENNYKTTPPVLDSDGSFFLYSKLTVDKSRWQQGNVFSCSVMHEALHNHYTQKSLSLSP

SEQ ID NO: 6 - protein, 214 aa, Artificial Sequence
  an artificially synthesized sequence
DIQMTQSPSSLSASVGDSVTITCQASQDISSYLNWYQQKPGKAPELLIYYGSELHSGVPSRFSGSGSGTDFTFTISSLEAEDAATYYCQQGNSLPYTFGQGTKVEIERTVAAPSVFIFPPSDEQLKSGTASVVCLLNNFYPREAKVQWKVDNALQSGNSQESVTEQDSKDSTYSLSSTLTLSKADYEKHKVYACEVTHQGLSSPVTKSFNRGEC

SEQ ID NO: 7 - protein, 453 aa, Artificial Sequence
  an artificially synthesized sequence
QVQLVQSGAEVKKPGSSVKVSCKASGGTFSSYAISWVRQAPGQGLEWMGGIIPIFGTANYAQKFQGRVTITADESTSTAYMELSSLRSEDTAVYYCARERDYYDSSGYYDAFDIWGQGTMVTVSSASTKGPSVFPLAPSSKSTSGGTAALGCLVKDYFPEPVTVSWNSGALTSGVHTFPAVLQSSGLYSLSSVVTVPSSSLGTQTYICNVNHKPSNTKVDKKVEPKSCDKTHTCPPCPAPELLGGPSVFLFPPKPKDTLMISRTPEVTCVVVDVSHEDPEVKFNWYVDGVEVHNAKTKPREEQYNSTYRVVSVLTVLHQDWLNGKEYKCKVSNKALPAPIEKTISKAKGQPREPQVYTLPPSRDELTKNQVSLTCLVKGFYPSDIAVEWESNGQPENNYKTTPPVLDSDGSFFLYSKLTVDKSRWQQGNVFSCSVMHEALHWHYTQKSLSLSP

SEQ ID NO: 8 - protein, 214 aa, Artificial Sequence; identical to SEQ ID NO: 4
  an artificially synthesized sequence

SEQ ID NO: 9 - protein, 449 aa, Artificial Sequence
  an artificially synthesized sequence
QVQLVQSGAEVKKPGASVKVSCKASGYTFTSYYMHWVRQAPGQGLEWMGIINPSGGSTSYAQKFQGRVTMTRDTSTSTVYMELSSLRSEDTAVYYCARDDPGGGEYYFDYWGQGTLVTVSSASTKGPSVFPLAPSSKSTSGGTAALGCLVKDYFPEPVTVSWNSGALTSGVHTFPAVLQSSGLYSLSSVVTVPSSSLGTQTYICNVNHKPSNTKVDKKVEPKSCDKTHTCPPCPAPELLGGPSVFLFPPKPKDTLMISRTPEVTCVVVDVSHEDPEVKFNWYVDGVEVHNAKTKPREEQYNSTYRVVSVLTVLHQDWLNGKEYKCKVSNKALPAPIEKTISKAKGQPREPQVYTLPPSRDELTKNQVSLTCLVKGFYPSDIAVEWESNGQPENNYKTTPPVLDSDGSFFLYSKLTVDKSRWQQGNVFSCSVMHEALHWHYTQKSLSLSP

SEQ ID NO: 10 - protein, 216 aa, Artificial Sequence; identical to SEQ ID NO: 2
  an artificially synthesized sequence

SEQ ID NO: 11 - protein, 447 aa, Artificial Sequence
  an artificially synthesized sequence
QVQLQESGPGLVKPSETLSLTCAVSGYSISDDQAWSWVRQPPGEGLEWIGYISYSGITNYNPSLKGRVTISRDTSKNQFSLKLSSVTAADTAAYYCARSLARTTAMDYWGEGTLVTVSSASTKGPSVFPLAPSSKSTSGGTAALGCLVKDYFPEPVTVSWNSGALTSGVHTFPAVLQSSGLYSLSSVVTVPSSSLGTQTYICNVNHKPSNTKVDKKVEPKSCDKTHTCPPCPAPELLGGPSVFLFPPKPKDTLMISRTPEVTCVVVDVSHEDPEVKFNWYVDGVEVHNAKTKPREEQYNSTYRVVSVLTVLHQDWLNGKEYKCKVSNKALPAPIEKTISKAKGQPREPQVYTLPPSRDELTKNQVSLTCLVKGFYPSDIAVEWESNGQPENNYKTTPPVLDSDGSFFLYSKLTVDKSRWQQGNVFSCSVMHEALHWHYTQKSLSLSP

SEQ ID NO: 12 - protein, 214 aa, Artificial Sequence; identical to SEQ ID NO: 6
  an artificially synthesized sequence

SEQ ID NO: 13 - protein, 449 aa, Artificial Sequence
  an artificially synthesized sequence
QVQLQESGPGLVRPSQTLSLTCTVSGYSITSDHAWSWVRQPPGRGLEWIGYISYSGITTYNPSLKSRVTMLRDTSKNQFSLRLSSVTAADTAVYYCARSLARTTAMDYWGQGSLVTVSSASTKGPSVFPLAPSSKSTSGGTAALGCLVKDYFPEPVTVSWNSGALTSGVHTFPAVLQSSGLYSLSSVVTVPSSSLGTQTYICNVNHKPSNTKVDKKVEPKSCDKTHTCPPCPAPELLGGPSVFLFPPKPKDTLMISRTPEVTCVVVDVSHEDPEVKFNWYVDGVEVHNAKTKPREEQYNSTYRVVSVLTVLHQDWLNGKEYKCKVSNKALPAPIEKTISKAKGQPREPQVYTLPPSRDELTKNQVSLTCLVKGFYPSDIAVEWESNGQPENNYKTTPPVLDSDGSFFLYSKLTVDKSRWQQGNVFSCSVMHEALHNHYTQKSLSLSPGK

SEQ ID NO: 14 - protein, 214 aa, Artificial Sequence [sequence omitted]

SEQ ID NO: 15 - protein, 468 aa, Homo sapiens
MLAVGCALLAALLAAPGAALAPRRCPAQEVARGVLTSLPGDSVTLTCPGVEPEDNATVHWVLRKPAAGSHPSRWAGMGRRLLLRSVQLHDSGNYSCYRAGRPAGTVHLLVDVPPEEPQLSCFRKSPLSNVVCEWGPRSTPSLTTKAVLLVRKFQNSPAEDFQEPCQYSQESQKFSCQLAVPEGDSSFYIVSMCVASSVGSKFSKTQTFQGCGILQPDPPANITVTAVARNPRWLSVTWQDPHSWNSSFYRLRFELRYRAERSKTFTTWMVKDLQHHCVIHDAWSGLRHVVQLRAQEEFGQGEWSEWSPEAMGTPWTESRSPPAENEVSTPMQALTTNKDDDNILFRDSANATSLPVQDSSSVPLPTFLVAGGSLAFGTLLCIAIVLRFKKTWKLRALKEGKTSMHPPYSLGQLVPERPRPTPVLVPLISPPVSPSSLGSDNTSSHNRPDARDPRSPYDISNTDYFFPR

SEQ ID NO: 16 - DNA, 1407 bp, Homo sapiens
atgctggccgtcggctgcgcgctgctggctgccctgctggccgcgccgggagcggcgctggccccaaggcgctgccctgcgcaggaggtggcgagaggcgtgctgaccagtctgccaggagacagcgtgactctgacctgcccgggggtagagccggaagacaatgccactgttcactgggtgctcaggaagccggctgcaggctcccaccccagcagatgggctggcatgggaaggaggctgctgctgaggtcggtgcagctccacgactctggaaactattcatgctaccgggccggccgcccagctgggactgtgcacttgctggtggatgttccccccgaggagccccagctctcctgcttccggaagagccccctcagcaatgttgtttgtgagtggggtcctcggagcaccccatccctgacgacaaaggctgtgctcttggtgaggaagtttcagaacagtccggccgaagacttccaggagccgtgccagtattcccaggagtcccagaagttctcctgccagttagcagtcccggagggagacagctctttctacatagtgtccatgtgcgtcgccagtagtgtcgggagcaagttcagcaaaactcaaacctttcagggttgtggaatcttgcagcctgatccgcctgccaacatcacagtcactgccgtggccagaaacccccgctggctcagtgtcacctggcaagacccccactcctggaactcatctttctacagactacggtttgagctcagatatcgggctgaacggtcaaagacattcacaacatggatggtcaaggacctccagcatcactgtgtcatccacgacgcctggagcggcctgaggcacgtggtgcagcttcgtgcccaggaggagttcgggcaaggcgagtggagcgagtggagcccggaggccatgggcacgccttggacagaatccaggagtcctccagctgagaacgaggtgtccacccccatgcaggcacttactactaataaagacgatgataatattctcttcagagattctgcaaatgcgacaagcctcccagtgcaagattcttcttcagtaccactgcccacattcctggttgctggagggagcctggccttcggaacgctcctctgcattgccattgttctgaggttcaagaagacgtggaagctgcgggctctgaaggaaggcaagacaagcatgcatccgccgtactctttggggcagctggtcccggagaggcctcgacccaccccagtgcttgttcctctcatctccccaccggtgtcccccagcagcctggggtctgacaatacctcgagccacaaccgaccagatgccagggacccacggagcccttatgacatcagcaatacagactacttcttccccagatag

SEQ ID NO: 17 - protein, 365 aa, Homo sapiens
MGVPRPQPWALGLLLFLLPGSLGAESHLSLLYHLTAVSSPAPGTPAFWVSGWLGPQQYLSYNSLRGEAEPCGAWVWENQVSWYWEKETTDLRIKEKLFLEAFKALGGKGPYTLQGLLGCELGPDNTSVPTAKFALNGEEFMNFDLKQGTWGGDWPEALAISQRWQQQDKAANKELTFLLFSCPHRLREHLERGRGNLEWKEPPSMRLKARPSSPGFSVLTCSAFSFYPPELQLRFLRNGLAAGTGQGDFGPNSDGSFHASSSLTVKSGDEHHYCCIVQHAGLAQPLRVELESPAKSSVLVVGIVIGVLLLTAAAVGGALLWRRMRSGLPAPWISLRGDDTGVLLPTPGEAQDADLKDVNVIPATA

SEQ ID NO: 18 - protein, 119 aa, Homo sapiens
MSRSVALAVLALLSLSGLEAIQRTPKIQVYSRHPAENGKSNFLNCYVSGFHPSDIEVDLLKNGERIEKVEHSDLSFSKDWSFYLLYYTEFTPTEKDEYACRVNHVTLSQPKIVKWDRDM

SEQ ID NO: 19 - protein, 447 aa, Homo sapiens
QVQLQESGPGLVKPSETLSLTCAVSGHSISHDHAWSWVRQPPGEGLEWIGFISYSGITNYNPSLQGRVTISRDNSKNTLYLQMNSLRAEDTAVYYCARSLARTTAMDYWGEGTLVTVSSASTKGPSVFPLAPSSKSTSGGTAALGCLVKDYFPEPVTVSWNSGALTSGVHTFPAVLQSSGLYSLSSVVTVPSSSLGTQTYICNVNHKPSNTKVDKKVEPKSCDKTHTCPPCPAPELLGGPSVFLFPPKPKDTLMISRTPEVTCVVVDVSHEDPEVKFNWYVDGVEVHNAKTKPREEQYNSTYRVVSVLTVLHQDWLNGKEYKCKVSNKALPAPIEKTISKAKGQPREPQVYTLPPSRDELTKNQVSLTCLVKGFYPSDIAVEWESNGQPENNYKTTPPVLDSDGSFFLYSKLTVDKSRWQQGNVFSCSVMHEALHNHYTQKSLSLSP

SEQ ID NO: 20 - protein, 214 aa, Homo sapiens
DIQMTQSPSSLSASVGDSVTITCQASTDISSHLNWYQQKPGKAPELLIYYGSHLLSGVPSRFSGSGSGTDFTFTISSLEAEDAATYYCGQGNRLPYTFGQGTKVEIERTVAAPSVFIFPPSDEQLKSGTASVVCLLNNFYPREAKVQWKVDNALQSGNSQESVTEQDSKDSTYSLSSTLTLSKADYEKHKVYACEVTHQGLSSPVTKSFNRGEC

SEQ ID NO: 21 - protein, 447 aa, Artificial Sequence
  an artificially synthesized sequence
QVQLQESGPGLVKPSETLSLTCAVSGHSISHDHAWSWVRQPPGEGLEWIGFISYSGITNYNPSLQGRVTISRDNSKNTLYLQMNSLRAEDTAVYYCARSLARTTAMDYWGEGTLVTVSSASTKGPSVFPLAPSSKSTSGGTAALGCLVKDYFPEPVTVSWNSGALTSGVHTFPAVLQSSGLYSLSSVVTVPSSSLGTQTYICNVNHKPSNTKVDKKVEPKSCDKTHTCPPCPAPELLGGPSVFLFPPKPKDTLYITREPEVTCVVVDVSHEDPEVKFNWYVDGVEVHNAKTKPREEQYNSTYRVVSVLTVLHQDWLNGKEYKCKVSNKALPAPIEKTISKAKGQPREPQVYTLPPSRDELTKNQVSLTCLVKGFYPSDIAVEWESNGQPENNYKTTPPVLDSDGSFFLYSKLTVDKSRWQQGNVFSCSVMHEALHNHYTQKSLSLSP

SEQ ID NO: 22 - protein, 447 aa, Artificial Sequence
  an artificially synthesized sequence
QVQLQESGPGLVKPSETLSLTCAVSGHSISHDHAWSWVRQPPGEGLEWIGFISYSGITNYNPSLQGRVTISRDNSKNTLYLQMNSLRAEDTAVYYCARSLARTTAMDYWGEGTLVTVSSASTKGPSVFPLAPSSKSTSGGTAALGCLVKDYFPEPVTVSWNSGALTSGVHTFPAVLQSSGLYSLSSVVTVPSSSLGTQTYICNVNHKPSNTKVDKKVEPKSCDKTHTCPPCPAPELLGGPSVFLFPPKPKDTLMISRTPEVTCVVVDVSHEDPEVKFNWYVDGVEVHNAKTKPREEQYNSTYRVVSVLTVLHQDWLNGKEYKCKVSNKALPAPIEKTISKAKGQPREPQVYTLPPSRDELTKNQVSLTCLVKGFYPSDIAVEWESNGQPENNYKTTPPVLDSDGSFFLYSKLTVDKSRWQQGNVFSCSVMHEALHWHYTQKSLSLSP

SEQ ID NO: 23 - protein, 447 aa, Artificial Sequence
  an artificially synthesized sequence
QVQLQESGPGLVKPSETLSLTCAVSGHSISHDHAWSWVRQPPGEGLEWIGFISYSGITNYNPSLQGRVTISRDNSKNTLYLQMNSLRAEDTAVYYCARSLARTTAMDYWGEGTLVTVSSASTKGPSVFPLAPSSKSTSGGTAALGCLVKDYFPEPVTVSWNSGALTSGVHTFPAVLQSSGLYSLSSVVTVPSSSLGTQTYICNVNHKPSNTKVDKKVEPKSCDKTHTCPPCPAPELLGGPSVFLFPPKPKDTLMISRTPEVTCVVVDVSHEDPEVKFNWYVDGVEVHNAKTKPREEQYNSTYRVVSVLTFLHQDWLNGKEYKCKVSNKALPAPIEKTISKAKGQPREPQVYTLPPSRDELTKNQVSLTCLVKGFYPSDIAVEWESNGQPENNYKTTPPVLDSDGSFFLYSKLTVDKSRWQQGNVFSCSVMHEALHYHYTQKSLSLSP

SEQ ID NO: 24 - protein, 443 aa, Artificial Sequence
  an artificially synthesized sequence
QVQLQESGPGLVKPSETLSLTCAVSGHSISHDHAWSWVRQPPGEGLEWIGFISYSGITNYNPSLQGRVTISRDNSKNTLYLQMNSLRAEDTAVYYCARSLARTTAMDYWGEGTLVTVSSASTKGPSVFPLAPSSKSTSGGTAALGCLVKDYFPEPVTVSWNSGALTSGVHTFPAVLQSSGLYSLSSVVTVPSSNFGTQTYTCNVDHKPSNTKVDKTVERKSCVECPPCPAPPVAGPSVFLFPPKPKDTLMISRTPEVTCVVVDVSQEDPEVQFNWYVDGVEVHNAKTKPREEQFNSTFRVVSVLTVVHQDWLNGKEYKCKVSNKGLPAPIEKTISKTKGQPREPQVYTLPPSQEEMTKNQVSLTCLVKGFYPSDIAVEWESNGQPENNYKTTPPMLDSDGSFFLYSKLTVDKSRWQEGNVFSCSVMHEALHAHYTQKSLSLSP

SEQ ID NO: 25 - protein, 126 aa, Artificial Sequence
  an artificially synthesized sequence
EVQLVESGGGLVQPGGSLRLSCAASGFTFSSYEMNWVRQAPGKGLEWVSYISSSGSTIYYADSVKGRFTISRDNAKNSLYLQMNSLRAEDTAVYYCARDAPYYYDSSGYTDAFDIWGQGTMVTVSS

SEQ ID NO: 26 - protein, 106 aa, Artificial Sequence
  an artificially synthesized sequence
EIVLTQSPATLSLSPGERATLSCRASQSVSSYLAWYQQKPGQAPRLLIFDASNRAAGIPARFSGSGSGTDFTLTISSLEPEDFAVYYCQQFDKWVTFGGGTTVEIR

SEQ ID NO: 27 - protein, 454 aa, Artificial Sequence
  an artificially synthesized sequence
EVQLVESGGGLVQPGGSLRLSCAASGFTFSSYEMNWVRQAPGKGLEWVSYISSSGSTIYYADSVKGRFTISRDNAKNSLYLQMNSLRAEDTAVYYCARDAPYYYDSSGYTDAFDIWGQGTMVTVSSASTKGPSVFPLAPSSKSTSGGTAALGCLVKDYFPEPVTVSWNSGALTSGVHTFPAVLQSSGLYSLSSVVTVPSSSLGTQTYICNVNHKPSNTKVDKKVEPKSCDKTHTCPPCPAPELLGGPSVFLFPPKPKDTLMISRTPEVTCVVVDVSHEDPEVKFNWYVDGVEVHNAKTKPREEQYNSTYRVVSVLTVLHQDWLNGKEYKCKVSNKALPAPIEKTISKAKGQPREPQVYTLPPSRDELTKNQVSLTCLVKGFYPSDIAVEWESNGQPENNYKTTPPVLDSDGSFFLYSKLTVDKSRWQQGNVFSCSVMHEALHNHYTQKSLSLSP

SEQ ID NO: 28 - protein, 107 aa, Artificial Sequence [sequence omitted]

SEQ ID NO: 29 - protein, 213 aa, Artificial Sequence
  an artificially synthesized sequence
EIVLTQSPATLSLSPGERATLSCRASQSVSSYLAWYQQKPGQAPRLLIFDASNRAAGIPARFSGSGSGTDFTLTISSLEPEDFAVYYCQQFDKWVTFGGGTTVEIRRTVAAPSVFIFPPSDEQLKSGTASVVCLLNNFYPREAKVQWKVDNALQSGNSQESVTEQDSKDSTYSLSSTLTLSKADYEKHKVYACEVTHQGLSSPVTKSFNRGEC

SEQ ID NO: 30 - protein, 454 aa, Artificial Sequence
  an artificially synthesized sequence
EVQLVESGGGLVQPGGSLRLSCAASGFTFSSYEMNWVRQAPGKGLEWVSYISSSGSTIYYAASVKGRFTISRDNAKNSLYLQMNSLRAEDTAVYYCARDAPYYYDSSGYTDAFDIWGQGTMVTVSSASTKGPSVFPLAPSSKSTSGGTAALGCLVKDYFPEPVTVSWNSGALTSGVHTFPAVLQSSGLYSLSSVVTVPSSSLGTQTYICNVNHKPSNTKVDKKVEPKSCDKTHTCPPCPAPELLGGPSVFLFPPKPKDTLMISRTPEVTCVVVDVSHEDPEVKFNWYVDGVEVHNAKTKPREEQYNSTYRVVSVLTVLHQDWLNGKEYKCKVSNKALPAPIEKTISKAKGQPREPQVYTLPPSRDELTKNQVSLTCLVKGFYPSDIAVEWESNGQPENNYKTTPPVLDSDGSFFLYSKLTVDKSRWQQGNVFSCSVMHEALHNHYTQKSLSLSP

SEQ ID NO: 31 - protein, 454 aa, Artificial Sequence
  an artificially synthesized sequence
EVQLVESGGGLVQPGGSLRLSCAASGFTFSSYEMNWVRQAPGKGLEWVSYISSSGSTIYYADSVKGRFTISRDNAKNSLYLQMNSLRAEDTAVYYCARAAPYYYDSSGYTDAFDIWGQGTMVTVSSASTKGPSVFPLAPSSKSTSGGTAALGCLVKDYFPEPVTVSWNSGALTSGVHTFPAVLQSSGLYSLSSVVTVPSSSLGTQTYICNVNHKPSNTKVDKKVEPKSCDKTHTCPPCPAPELLGGPSVFLFPPKPKDTLMISRTPEVTCVVVDVSHEDPEVKFNWYVDGVEVHNAKTKPREEQYNSTYRVVSVLTVLHQDWLNGKEYKCKVSNKALPAPIEKTISKAKGQPREPQVYTLPPSRDELTKNQVSLTCLVKGFYPSDIAVEWESNGQPENNYKTTPPVLDSDGSFFLYSKLTVDKSRWQQGNVFSCSVMHEALHNHYTQKSLSLSP

SEQ ID NO: 32 - protein, 454 aa, Artificial Sequence
  an artificially synthesized sequence
EVQLVESGGGLVQPGGSLRLSCAASGFTFSSYEMNWVRQAPGKGLEWVSYISSSGSTIYYADSVKGRFTISRDNAKNSLYLQMNSLRAEDTAVYYCARDAPYYYASSGYTDAFDIWGQGTMVTVSSASTKGPSVFPLAPSSKSTSGGTAALGCLVKDYFPEPVTVSWNSGALTSGVHTFPAVLQSSGLYSLSSVVTVPSSSLGTQTYICNVNHKPSNTKVDKKVEPKSCDKTHTCPPCPAPELLGGPSVFLFPPKPKDTLMISRTPEVTCVVVDVSHEDPEVKFNWYVDGVEVHNAKTKPREEQYNSTYRVVSVLTVLHQDWLNGKEYKCKVSNKALPAPIEKTISKAKGQPREPQVYTLPPSRDELTKNQVSLTCLVKGFYPSDIAVEWESNGQPENNYKTTPPVLDSDGSFFLYSKLTVDKSRWQQGNVFSCSVMHEALHNHYTQKSLSLSP

SEQ ID NO: 33 - protein, 454 aa, Artificial Sequence
  an artificially synthesized sequence
EVQLVESGGGLVQPGGSLRLSCAASGFTFSSYEMNWVRQAPGKGLEWVSYISSSGSTIYYADSVKGRFTISRDNAKNSLYLQMNSLRAEDTAVYYCARDAPYYYDSSGYTAAFDIWGQGTMVTVSSASTKGPSVFPLAPSSKSTSGGTAALGCLVKDYFPEPVTVSWNSGALTSGVHTFPAVLQSSGLYSLSSVVTVPSSSLGTQTYICNVNHKPSNTKVDKKVEPKSCDKTHTCPPCPAPELLGGPSVFLFPPKPKDTLMISRTPEVTCVVVDVSHEDPEVKFNWYVDGVEVHNAKTKPREEQYNSTYRVVSVLTVLHQDWLNGKEYKCKVSNKALPAPIEKTISKAKGQPREPQVYTLPPSRDELTKNQVSLTCLVKGFYPSDIAVEWESNGQPENNYKTTPPVLDSDGSFFLYSKLTVDKSRWQQGNVFSCSVMHEALHNHYTQKSLSLSP

SEQ ID NO: 34 - protein, 454 aa, Artificial Sequence
  an artificially synthesized sequence
EVQLVESGGGLVQPGGSLRLSCAASGFTFSSYEMNWVRQAPGKGLEWVSYISSSGSTIYYADSVKGRFTISRDNAKNSLYLQMNSLRAEDTAVYYCARDAPYYYDSSGYTDAFAIWGQGTMVTVSSASTKGPSVFPLAPSSKSTSGGTAALGCLVKDYFPEPVTVSWNSGALTSGVHTFPAVLQSSGLYSLSSVVTVPSSSLGTQTYICNVNHKPSNTKVDKKVEPKSCDKTHTCPPCPAPELLGGPSVFLFPPKPKDTLMISRTPEVTCVVVDVSHEDPEVKFNWYVDGVEVHNAKTKPREEQYNSTYRVVSVLTVLHQDWLNGKEYKCKVSNKALPAPIEKTISKAKGQPREPQVYTLPPSRDELTKNQVSLTCLVKGFYPSDIAVEWESNGQPENNYKTTPPVLDSDGSFFLYSKLTVDKSRWQQGNVFSCSVMHEALHNHYTQKSLSLSP

SEQ ID NO: 35 - protein, 213 aa, Artificial Sequence
  an artificially synthesized sequence
EIVLTQSPATLSLSPGERATLSCRASQSVSSYLAWYQQKPGQAPRLLIFAASNRAAGIPARFSGSGSGTDFTLTISSLEPEDFAVYYCQQFDKWVTFGGGTTVEIRRTVAAPSVFIFPPSDEQLKSGTASVVCLLNNFYPREAKVQWKVDNALQSGNSQESVTEQDSKDSTYSLSSTLTLSKADYEKHKVYACEVTHQGLSSPVTKSFNRGEC

SEQ ID NO: 36 - protein, 213 aa, Artificial Sequence
  an artificially synthesized sequence
EIVLTQSPATLSLSPGERATLSCRASQSVSSYLAWYQQKPGQAPRLLIFDASNRAAGIPARFSGSGSGTDFTLTISSLEPEDFAVYYCQQFAKWVTFGGGTTVEIRRTVAAPSVFIFPPSDEQLKSGTASVVCLLNNFYPREAKVQWKVDNALQSGNSQESVTEQDSKDSTYSLSSTLTLSKADYEKHKVYACEVTHQGLSSPVTKSFNRGEC

SEQ ID NO: 37 - protein, 107 aa, Artificial Sequence
  an artificially synthesized sequence
DIQMTQSPSSLSASVGDRVTITCRASQSISSYLNWYQQKPGKAPKLLIYAASSLQSGVPSRFSGSGSGTDFTLTISSLQPEDFATYYCQQSYSTPFTFGPGTKVDIK

SEQ ID NO: 38 - protein, 112 aa, Artificial Sequence
  an artificially synthesized sequence
DIVMTQSPLSLPVTPGEPASISCRSSQSLLHSNGDNYLDWYLQKPGQSPQLLIYLGSNRASGVPDRFSGSGSGTDFTLKISRVEAEDVGVYYCMQVLRNPLTFGGGTKVEIQ

SEQ ID NO: 39 - protein, 107 aa, Artificial Sequence
  an artificially synthesized sequence
EIVMTQSPATLSLSPGERATLSCRASQSVSSYLAWYQQKPGQAPRLLIYDASNRATGIPARFSGSGSGTDFTLTISSLEPEDFAVYYCQQRSNWPPTFGQGTKVEIK

SEQ ID NO: 40 - protein, 112 aa, Artificial Sequence
  an artificially synthesized sequence
DIVMTQSPESLVLSLGGTATINCRSSQSVLYSSNNKNYLTWYQQKPGQPPTLLFSWASIRDSGVPDRFSASGSGTEFTLTISDLQAEDAAVYYCQQYYRAPSFGQGTKLQIK

SEQ ID NO: 41 - protein, 107 aa, Artificial Sequence
  an artificially synthesized sequence
ETTLTQSPAFMSATPGDKVNISCKASQDIDDDMNWYQQKPGEAAIFIIQEATTLVPGISPRFSGSGYGTDFTLTINNIESEDAAYYFCLQHDNFPYTFGQGTKLEIK

SEQ ID NO: 42 - protein, 128 aa, Artificial Sequence
  an artificially synthesized sequence
QVQLVQSGAEVKKPGASVKVSCKASGYTFTSYYMHWVRQAPGQGLEWMGIINPSGGSTSYAQKFQGRVTMTRDTSTSTVYMELSSLRSEDTAVYYCARDGTLYDFWSGYYSYDAFDIWGQGTMVTVSS

SEQ ID NO: 43 - protein, 122 aa, Artificial Sequence
  an artificially synthesized sequence
QMQLVQSGAEVKKPGSSVKVSCKASGGTFSSYAISWVRQAPGQGLEWMGGIIPIFGTANYAQKFQGRVTITADESTSTAYMELSSLRSEDTAVYYCARDLDTGPYYYGMDVWGQGTMVTVSS

SEQ ID NO: 44 - protein, 124 aa, Artificial Sequence
  an artificially synthesized sequence
QVQLVQSGAEVKKPGSSVKVSCKASGGTFSSYAISWVRQAPGQGLEWMGGIIPIFGTANYAQKFQGRVTITADESTSTAYMELSSLRSEDTAVYYCARDSPVPGVYYYYGMDVWGQGTMVTVSS

SEQ ID NO: 45 - protein, 119 aa, Artificial Sequence
  an artificially synthesized sequence
QVQLVQSGAEVKKPGESLKISCKGSGYSFTSYWIGWVRQMPGKGLEWMGIIYPGDSDTRYSPSFQGQVTISADKSISTAYLQWSSLKASDTAMYYCARHRAGDLGGDYWGQGTLVTVSS

SEQ ID NO: 46 - protein, 121 aa, Artificial Sequence
  an artificially synthesized sequence
QVQLVQSGAEVKKPGASVKVSCKASGYTFTGYIMNWVRQAPGQGLEWMGLINPYNGGTDYNPQFQDRVTITADKSTSTAYMELSSLRSEDTAVYYCARDGYDDGPYTLETWGQGTLVTVSS

SEQ ID NO: 47 - protein, 214 aa, Artificial Sequence
  an artificially synthesized sequence
ETTLTQSPAFMSATPGDKVTISCKASQDIDDDMNWYQQKPGEAAIFIIQEATTLVPGISPRFSGSGYGTDFTLTINNIESEDAAYYFCLQHDNFPYTFGQGTKLEIKRTVAAPSVFIFPPSDEQLKSGTASVVCLLNNFYPREAKVQWKVDNALQSGNSQESVTEQDSKDSTYSLSSTLTLSKADYEKHKVYACEVTHQGLSSPVTKSFNRGEC

SEQ ID NO: 48 - protein, 445 aa, Artificial Sequence
  an artificially synthesized sequence
QVQLVQSGAEVKKPGASVKVSCKASGYTFTGYIMNWVRQAPGQGLEWMGLINPYNGGTDYNPQFQDRVTITADKSTSTAYMELSSLRSEDTAVYYCARDGYDDGPYTLETWGQGTLVTVSSASTKGPSVFPLAPSSKSTSGGTAALGCLVKDYFPEPVTVSWNSGALTSGVHTFPAVLQSSGLYSLSSVVTVPSSNFGTQTYTCNVDHKPSNTKVDKTVERKSCVECPPCPAPPVAGPSVFLFPPKPKDTLMISRTPEVTCVVVDVSQEDPEVQFNWYVDGVEVHNAKTKPREEQFNSTFRVVSVLTVVHQDWLNGKEYKCKVSNKGLPAPIEKTISKTKGQPREPQVYTLPPSQEEMTKNQVSLTCLVKGFYPSDIAVEWESNGQPENNYKTTPPMLDSDGSFFLYSKLTVDKSRWQEGNVFSCSVMHEALHNHYTQKSLSLSP

SEQ ID NO: 49 - protein, 107 aa, Artificial Sequence
  an artificially synthesized sequence
DIQMTQSPSSLSASVGDRVTITCKASQDIDDDMNWYQQKPGKAPKLLIYEATTLVPGVPSRFSGSGSGTDFTLTISSLQPEDFATYYCLQHDNFPYTFGQGTKVEIK

SEQ ID NO: 50 - protein, 107 aa, Artificial Sequence
  an artificially synthesized sequence
DIVMTQSPLSLPVTPGEPASISCKASQDIDDDMNWYLQKPGQSPQLLIYEATTLVPGVPDRFSGSGSGTDFTLKISRVEAEDVGVYYCLQHDNFPYTFGQGTKLEIK

SEQ ID NO: 51 - protein, 107 aa, Artificial Sequence
  an artificially synthesized sequence
EIVLTQSPGTLSLSPGERATLSCKASQDIDDDMNWYQQKPGQAPRLLIYEATTLVPGIPDRFSGSGSGTDFTLTISRLEPEDFAVYYCLQHDNFPYTFGQGTKVEIK

SEQ ID NO: 52 - protein, 107 aa, Artificial Sequence
  an artificially synthesized sequence
DIVMTQSPDSLAVSLGERATINCKASQDIDDDMNWYQQKPGQPPKLLIYEATTLVPGVPDRFSGSGSGTDFTLTISSLQAEDVAVYYCLQHDNFPYTFGQGTKLEIK

SEQ ID NO: 53 - protein, 214 aa, Artificial Sequence
  an artificially synthesized sequence
ETTLTQSPAFMSATPGDKVTISCKASQDIADDMNWYQQKPGEAAIFIIQEATTLVPGISPRFSGSGYGTDFTLTINNIESEDAAYYFCLQHDNFPYTFGQGTKLEIKRTVAAPSVFIFPPSDEQLKSGTASVVCLLNNFYPREAKVQWKVDNALQSGNSQESVTEQDSKDSTYSLSSTLTLSKADYEKHKVYACEVTHQGLSSPVTKSFNRGEC

SEQ ID NO: 54 - protein, 214 aa, Artificial Sequence
  an artificially synthesized sequence
ETTLTQSPAFMSATPGDKVTISCKASQDIDADMNWYQQKPGEAAIFIIQEATTLVPGISPRFSGSGYGTDFTLTINNIESEDAAYYFCLQHDNFPYTFGQGTKLEIKRTVAAPSVFIFPPSDEQLKSGTASVVCLLNNFYPREAKVQWKVDNALQSGNSQESVTEQDSKDSTYSLSSTLTLSKADYEKHKVYACEVTHQGLSSPVTKSFNRGEC

SEQ ID NO: 55 - protein, 214 aa, Artificial Sequence
  an artificially synthesized sequence
ETTLTQSPAFMSATPGDKVTISCKASQDIDDAMNWYQQKPGEAAIFIIQEATTLVPGISPRFSGSGYGTDFTLTINNIESEDAAYYFCLQHDNFPYTFGQGTKLEIKRTVAAPSVFIFPPSDEQLKSGTASVVCLLNNFYPREAKVQWKVDNALQSGNSQESVTEQDSKDSTYSLSSTLTLSKADYEKHKVYACEVTHQGLSSPVTKSFNRGEC

SEQ ID NO: 56 - protein, 214 aa, Artificial Sequence
  an artificially synthesized sequence
ETTLTQSPAFMSATPGDKVTISCKASQDIDDDMNWYQQKPGEAAIFIIQAATTLVPGISPRFSGSGYGTDFTLTINNIESEDAAYYFCLQHDNFPYTFGQGTKLEIKRTVAAPSVFIFPPSDEQLKSGTASVVCLLNNFYPREAKVQWKVDNALQSGNSQESVTEQDSKDSTYSLSSTLTLSKADYEKHKVYACEVTHQGLSSPVTKSFNRGEC

SEQ ID NO: 57 - protein, 214 aa, Artificial Sequence
  an artificially synthesized sequence
ETTLTQSPAFMSATPGDKVTISCKASQDIADAMNWYQQKPGEAAIFIIQEATTLVPGISPRFSGSGYGTDFTLTINNIESEDAAYYFCLQHDNFPYTFGQGTKLEIKRTVAAPSVFIFPPSDEQLKSGTASVVCLLNNFYPREAKVQWKVDNALQSGNSQESVTEQDSKDSTYSLSSTLTLSKADYEKHKVYACEVTHQGLSSPVTKSFNRGEC

SEQ ID NO: 58 - protein, 214 aa, Artificial Sequence
  an artificially synthesized sequence
ETTLTQSPAFMSATPGDKVTISCKASQDIADDMNWYQQKPGEAAIFIIQAATTLVPGISPRFSGSGYGTDFTLTINNIESEDAAYYFCLQHDNFPYTFGQGTKLEIKRTVAAPSVFIFPPSDEQLKSGTASVVCLLNNFYPREAKVQWKVDNALQSGNSQESVTEQDSKDSTYSLSSTLTLSKADYEKHKVYACEVTHQGLSSPVTKSFNRGEC

SEQ ID NO: 59 - protein, 214 aa, Artificial Sequence
  an artificially synthesized sequence
ETTLTQSPAFMSATPGDKVTISCKASQDIADAMNWYQQKPGEAAIFIIQAATTLVPGISPRFSGSGYGTDFTLTINNIESEDAAYYFCLQHDNFPYTFGQGTKLEIKRTVAAPSVFIFPPSDEQLKSGTASVVCLLNNFYPREAKVQWKVDNALQSGNSQESVTEQDSKDSTYSLSSTLTLSKADYEKHKVYACEVTHQGLSSPVTKSFNRGEC

SEQ ID NO: 60 - protein, 214 aa, Artificial Sequence
  an artificially synthesized sequence
ETTLTQSPAFMSATPGDKVTISCKASQDIDDDMNWYQQKPGEAAIFIIQEATTLVPGISPRFSGSGYGTDFTLTINNIESEDAAYYFCLQHANFPYTFGQGTKLEIKRTVAAPSVFIFPPSDEQLKSGTASVVCLLNNFYPREAKVQWKVDNALQSGNSQESVTEQDSKDSTYSLSSTLTLSKADYEKHKVYACEVTHQGLSSPVTKSFNRGEC

SEQ ID NO: 61 - protein, 214 aa, Artificial Sequence
  an artificially synthesized sequence
DIQMTQSPSSLSASVGDRVTITCRASQSIDDDLNWYQQKPGKAPKLLIYEASSLQSGVPSRFSGSGSGTDFTLTISSLQPEDFATYYCQQSDSTPYTFGQGTKVEIKRTVAAPSVFIFPPSDEQLKSGTASVVCLLNNFYPREAKVQWKVDNALQSGNSQESVTEQDSKDSTYSLSSTLTLSKADYEKHKVYACEVTHQGLSSPVTKSFNRGEC

SEQ ID NO: 62 - protein, 214 aa, Artificial Sequence
  an artificially synthesized sequence
DIQMTQSPSSLSASVGDRVTITCRASQSISSYLNWYQQKPGKAPKLLIYAASSLQSGVPSRFSGSGSGTDFTLTISSLQPEDFATYYCQQSYSTPYTFGQGTKVEIKRTVAAPSVFIFPPSDEQLKSGTASVVCLLNNFYPREAKVQWKVDNALQSGNSQESVTEQDSKDSTYSLSSTLTLSKADYEKHKVYACEVTHQGLSSPVTKSFNRGEC

SEQ ID NO: 63 - protein, 214 aa, Artificial Sequence
  an artificially synthesized sequence
ETTLTQSPAFMSATPGDKVNISCKASQDIDDDMNWYQQKPGEAAIFIIQEATTLVPGIPPRFSGSGYGTDFTLTINNIESEDAAYYFCLQHDNFPLTFGQGTKVEIKRTVAAPSVFIFPPSDEQLKSGTASVVCLLNNFYPREAKVQWKVDNALQSGNSQESVTEQDSKDSTYSLSSTLTLSKADYEKHKVYACEVTHQGLSSPVTKSFNRGEC

SEQ ID NO: 64 - protein, 214 aa, Artificial Sequence
  an artificially synthesized sequence
ETTLTQSPAFMSATPGDKVNISCKASQDIEDDMNWYQQKPGEAAIFIIQEATTLVPGISPRFSGSGYGTDFTLTINNIESEDAAYYFCLQHDNFPLTFGQGTKVEIKRTVAAPSVFIFPPSDEQLKSGTASVVCLLNNFYPREAKVQWKVDNALQSGNSQESVTEQDSKDSTYSLSSTLTLSKADYEKHKVYACEVTHQGLSSPVTKSFNRGEC

SEQ ID NO: 65 - protein, 328 aa, Artificial Sequence
  an artificially synthesized sequence
ASTKGPSVFPLAPSSKSTSGGTAALGCLVKDYFPEPVTVSWNSGALTSGVHTFPAVLQSSGLYSLSSVVTVPSSSLGTQTYICNVNHKPSNTKVDKKVEPKSCDKTHTCPPCPAPELLGGPSVFLFPPKPKDTLMISRTPEVTCVVVDVSHEDPEVKFNWYVDGVEVHNAKTKPREEQYNSTYRVVSVLTVLHQDWLNGKEYKCKVSNKALPAPIEKTISKAKGQPREPQVYTLPPSRDELTKNQVSLTCLVKGFYPSDIAVEWESNGQPENNYKTTPPVLDSDGSFFLYSKLTVDKSRWQQGNVFSCSVMHEALHNHYTQKSLSLSP

SEQ ID NO: 66 - protein, 462 aa, Artificial Sequence
  an artificially synthesized sequence
QVQLVQSGAEVKKPGSSVKVSCKASGGTFSSYAISWVRQAPGQGLEWMGGIIPIFGTANYAQKFQGRVTITADESTSTAYMELSSLRSEDTAVYYCARDLGDIVVVPAAPDMPKGYYYYGMDVWGQGTMVTVSSASTKGPSVFPLAPSSKSTSGGTAALGCLVKDYFPEPVTVSWNSGALTSGVHTFPAVLQSSGLYSLSSVVTVPSSSLGTQTYICNVNHKPSNTKVDKKVEPKSCDKTHTCPPCPAPELLGGPSVFLFPPKPKDTLMISRTPEVTCVVVDVSHEDPEVKFNWYVDGVEVHNAKTKPREEQYNSTYRVVSVLTVLHQDWLNGKEYKCKVSNKALPAPIEKTISKAKGQPREPQVYTLPPSRDELTKNQVSLTCLVKGFYPSDIAVEWESNGQPENNYKTTPPVLDSDGSFFLYSKLTVDKSRWQQGNVFSCSVMHEALHNHYTQKSLSLSP

SEQ ID NO: 67 - protein, 215 aa, Artificial Sequence
  an artificially synthesized sequence
EIVMTQSPATLSVSPGERATLSCRASQSINDNLAWYQQKPGQAPRLLIYGASTRATGIPARFSGSGSGTEFTLTISSLQSEDFAVYFCQQYQYWPPITFGQGTRLDIKRTVAAPSVFIFPPSDEQLKSGTASVVCLLNNFYPREAKVQWKVDNALQSGNSQESVTEQDSKDSTYSLSSTLTLSKADYEKHKVYACEVTHQGLSSPVTKSFNRGEC

SEQ ID NO: 68 - protein, 446 aa, Artificial Sequence
  an artificially synthesized sequence
QVQLVQSGAEVKKPGATVKISCKVSGYTFTDYYMHWVQQAPGKGLEWMGLVDPEDGETIYAEKFQGRVTITADTSTDTAYMELSSLRSEDTAVYYCATAGSSSNFDYWGQGTLVTVSSASTKGPSVFPLAPSSKSTSGGTAALGCLVKDYFPEPVTVSWNSGALTSGVHTFPAVLQSSGLYSLSSVVTVPSSSLGTQTYICNVNHKPSNTKVDKKVEPKSCDKTHTCPPCPAPELLGGPSVFLFPPKPKDTLMISRTPEVTCVVVDVSHEDPEVKFNWYVDGVEVHNAKTKPREEQYNSTYRVVSVLTVLHQDWLNGKEYKCKVSNKALPAPIEKTISKAKGQPREPQVYTLPPSRDELTKNQVSLTCLVKGFYPSDIAVEWESNGQPENNYKTTPPVLDSDGSFFLYSKLTVDKSRWQQGNVFSCSVMHEALHNHYTQKSLSLSP

SEQ ID NO: 69 - protein, 216 aa, Artificial Sequence
  an artificially synthesized sequence
QSALTQPRSVSGSPGQSVTISCTGTSSDVGGYNYVSWYQQHPGKAPKLMIYDVSKRPSGVPDRFSGSKSGNTASLTISGLQAEDEADYYCCSYAGSYTWVFGGGTKLTVLGQPKAAPSVTLFPPSSEELQANKATLVCLISDFYPGAVTVAWKADSSPVKAGVETTTPSKQSNNKYAASSYLSLTPEQWKSHRSYSCQVTHEGSTVEKTVAPTECS

SEQ ID NO: 70 - protein, 452 aa, Artificial Sequence
  an artificially synthesized sequence
QVQLQQSGPGLVKPSQTLSLTCAISGDSVSSNSAAWNWIRQSPSRGLEWLGRTYYRSKWYNDYAVSVKSRITINPDTSKNQFSLQLNSVTPEDTAVYYCARDLIAAAGGDFDYWGQGTLVTVSSASTKGPSVFPLAPSSKSTSGGTAALGCLVKDYFPEPVTVSWNSGALTSGVHTFPAVLQSSGLYSLSSVVTVPSSSLGTQTYICNVNHKPSNTKVDKKVEPKSCDKTHTCPPCPAPELLGGPSVFLFPPKPKDTLMISRTPEVTCVVVDVSHEDPEVKFNWYVDGVEVHNAKTKPREEQYNSTYRVVSVLTVLHQDWLNGKEYKCKVSNKALPAPIEKTISKAKGQPREPQVYTLPPSRDELTKNQVSLTCLVKGFYPSDIAVEWESNGQPENNYKTTPPVLDSDGSFFLYSKLTVDKSRWQQGNVFSCSVMHEALHNHYTQKSLSLSP

SEQ ID NO: 71 - protein, 217 aa, Artificial Sequence
  an artificially synthesized sequence
QSVLTQPPSVSGAPGQRVTISCTGSRSNIGAGFDVHWYRQLPGTAPKLLIYGISNRPSGVPDRFSGSKSDTSVSLAITGLQAEDEADYYCQSYDSSLSGYVFGTGTKVTVLGQPKANPTVTLFPPSSEELQANKATLVCLISDFYPGAVTVAWKADGSPVKAGVETTKPSKQSNNKYAASSYLSLTPEQWKSHRSYSCQVTHEGSTVEKTVAPTECS

SEQ ID NO: 72 - protein, 214 aa, Artificial Sequence
  an artificially synthesized sequence
DIQMTQSPSSLSASVGDRVTITCRASQSIADDLNWYQQKPGKAPKLLIYEASSLQSGVPSRFSGSGSGTDFTLTISSLQPEDFATYYCQQSDSTPYTFGQGTKVEIKRTVAAPSVFIFPPSDEQLKSGTASVVCLLNNFYPREAKVQWKVDNALQSGNSQESVTEQDSKDSTYSLSSTLTLSKADYEKHKVYACEVTHQGLSSPVTKSFNRGEC

SEQ ID NO: 73 - protein, 214 aa, Artificial Sequence
  an artificially synthesized sequence
DIQMTQSPSSLSASVGDRVTITCRASQSIDADLNWYQQKPGKAPKLLIYEASSLQSGVPSRFSGSGSGTDFTLTISSLQPEDFATYYCQQSDSTPYTFGQGTKVEIKRTVAAPSVFIFPPSDEQLKSGTASVVCLLNNFYPREAKVQWKVDNALQSGNSQESVTEQDSKDSTYSLSSTLTLSKADYEKHKVYACEVTHQGLSSPVTKSFNRGEC

SEQ ID NO: 74 - protein, 214 aa, Artificial Sequence
  an artificially synthesized sequence
DIQMTQSPSSLSASVGDRVTITCRASQSIDDALNWYQQKPGKAPKLLIYEASSLQSGVPSRFSGSGSGTDFTLTISSLQPEDFATYYCQQSDSTPYTFGQGTKVEIKRTVAAPSVFIFPPSDEQLKSGTASVVCLLNNFYPREAKVQWKVDNALQSGNSQESVTEQDSKDSTYSLSSTLTLSKADYEKHKVYACEVTHQGLSSPVTKSFNRGEC

SEQ ID NO: 75 - protein, 214 aa, Artificial Sequence
  an artificially synthesized sequence
DIQMTQSPSSLSASVGDRVTITCRASQSISDDLNWYQQKPGKAPKLLIYEASSLQSGVPSRFSGSGSGTDFTLTISSLQPEDFATYYCQQSDSTPYTFGQGTKVEIKRTVAAPSVFIFPPSDEQLKSGTASVVCLLNNFYPREAKVQWKVDNALQSGNSQESVTEQDSKDSTYSLSSTLTLSKADYEKHKVYACEVTHQGLSSPVTKSFNRGEC

SEQ ID NO: 76 - protein, 383 aa, Artificial Sequence
  an artificially synthesized sequence
KKVVLGKKGDTVELTCTASQKKSIQFHWKNSNQIKILGNQGSFLTKGPSKLNDRADSRRSLWDQGNFPLIIKNLKIEDSDTYICEVEDQKEEVQLLVFGLTANSDTHLLQGQSLTLTLESPPGSSPSVQCRSPRGKNIQGGKTLSVSQLELQDSGTWTCTVLQNQKKVEFKIDIVVLAFQKASSIVYKKEGEQVEFSFPLAFTVEKLTGSGELWWQAERASSSKSWITFDLKNKEVSVKRVTQDPKLQMGKKLPLHLTLPQALPQYAGSGNLTLALEAKTGKLHQEVNLVVMRATQLQKNLTCEVWGPTSPKLMLSLKLENKEAKVSKREKAVWVLNPEAGMWQCLLSDSGQVLLESNIKVLPTWEQKLISEEDLDYKDDDDK

SEQ ID NO: 77 - protein, 450 aa, Artificial Sequence
  an artificially synthesized sequence
QVQLQQSGPEVVKPGASVKMSCKASGYTFTSYVIHWVRQKPGQGLDWIGYINPYNDGTDYDEKFKGKATLTSDTSTSTAYMELSSLRSEDTAVYYCAREKDNYATGAWFAYWGQGTLVTVSSASTKGPSVFPLAPSSKSTSGGTAALGCLVKDYFPEPVTVSWNSGALTSGVHTFPAVLQSSGLYSLSSVVTVPSSSLGTQTYICNVNHKPSNTKVDKKVEPKSCDKTHTCPPCPAPELLGGPSVFLFPPKPKDTLMISRTPEVTCVVVDVSHEDPEVKFNWYVDGVEVHNAKTKPREEQYNSTYRVVSVLTVLHQDWLNGKEYKCKVSNKALPAPIEKTISKAKGQPREPQVYTLPPSRDELTKNQVSLTCLVKGFYPSDIAVEWESNGQPENNYKTTPPVLDSDGSFFLYSKLTVDKSRWQQGNVFSCSVMHEALHNHYTQKSLSLSP

SEQ ID NO: 78 - protein, 219 aa, Artificial Sequence
  an artificially synthesized sequence
DIVMTQSPDSLAVSLGERVTMNCKSSQSLLYSTNQKNYLAWYQQKPGQSPKLLIYWASTRESGVPDRFSGSGSGTDFTLTISSVQAEDVAVYYCQQYYSYRTFGGGTKLEIKRTVAAPSVFIFPPSDEQLKSGTASVVCLLNNFYPREAKVQWKVDNALQSGNSQESVTEQDSKDSTYSLSSTLTLSKADYEKHKVYACEVTHQGLSSPVTKSFNRGEC

SEQ ID NO: 79 - protein, 448 aa, Artificial Sequence
  an artificially synthesized sequence
EVQLVESGGDLVKPGGSLKLSCAASGFTFSSYGMSWVRQTPDKGLEWVATISSGGSYTYYPDNVKGRFTISRDNAKNTLYLQMSSLKSEDTAMYYCARHEDGNWNYFDYWGQGTTLTVSSASTKGPSVFPLAPSSKSTSGGTAALGCLVKDYFPEPVTVSWNSGALTSGVHTFPAVLQSSGLYSLSSVVTVPSSSLGTQTYICNVNHKPSNTKVDKKVEPKSCDKTHTCPPCPAPELLGGPSVFLFPPKPKDTLMISRTPEVTCVVVDVSHEDPEVKFNWYVDGVEVHNAKTKPREEQYNSTYRVVSVLTVLHQDWLNGKEYKCKVSNKALPAPIEKTISKAKGQPREPQVYTLPPSRDELTKNQVSLTCLVKGFYPSDIAVEWESNGQPENNYKTTPPVLDSDGSFFLYSKLTVDKSRWQQGNVFSCSVMHEALHNHYTQKSLSLSP

SEQ ID NO: 80 - protein, 214 aa, Artificial Sequence
  an artificially synthesized sequence
ETTVTQSPASLSVAIGEKVTIRCITSTDIDDDMNWYQQKPGEPPKFFISEGNTLRPGVPSRFSSSGYGTDFVFTIENMLSEDVADYYCLQSDTLPLTFGSGTKLEIKRTVAAPSVFIFPPSDEQLKSGTASVVCLLNNFYPREAKVQWKVDNALQSGNSQESVTEQDSKDSTYSLSSTLTLSKADYEKHKVYACEVTHQGLSSPVTKSFNRGEC

SEQ ID NO: 81 - protein, 448 aa, Artificial Sequence; identical to SEQ ID NO: 79
  an artificially synthesized sequence

SEQ ID NO: 82 - protein, 214 aa, Artificial Sequence
  an artificially synthesized sequence
ETTVTQSPASLSVAIGEKVTIRCITSTDIDDDMNWYQQKPGEPPKFFISNGNTLRPGVPSRFSSSGYGTDFVFTIENMLSEDVADYYCLQSDTLPLTFGSGTKLEIKRTVAAPSVFIFPPSDEQLKSGTASVVCLLNNFYPREAKVQWKVDNALQSGNSQESVTEQDSKDSTYSLSSTLTLSKADYEKHKVYACEVTHQGLSSPVTKSFNRGEC

SEQ ID NO: 83 - protein, 464 aa, Artificial Sequence
  an artificially synthesized sequence
QVQLQESGPGLVRPSQTLSLTCTVSGYSITSDHAWSWVRQPPGRGLEWIGYISYSGITTYNPSLKSRVTMLRDTSKNQFSLRLSSVTAADTAVYYCARSLARTTAMDYWGQGSLVTVSSASPTSPKVFPLSLCSTQPDGNVVIACLVQGFFPQEPLSVTWSESGQGVTARNFPPSQDASGDLYTTSSQLTLPATQCLAGKSVTCHVKHYTNPSQDVTVPCPVPSTPPTPSPSTPPTPSPSCCHPRLSLHRPALEDLLLGSEANLTCTLTGLRDASGVTFTWTPSSGKSAVQGPPERDLCGCYSVSSVLPGCAEPWNHGKTFTCTAAYPESKTPLTATLSKSGNTFRPEVHLLPPPSEELALNELVTLTCLARGFSPKDVLVRWLQGSQELPREKYLTWASRQEPSQGTTTFAVTSILRVAAEDWKKGDTFSCMVGHEALPLAFTQKTIDRLAGKEQKLISEEDL

SEQ ID NO: 84 - protein, 450 aa, Artificial Sequence
  an artificially synthesized sequence
EVQLVQSGAEVKKPGSSVKVSCKASGGTFSSYAISWVRQAPGQGLEWMGGIIPIFGTANYAQKFQGRVTITADESTSTAYMELSSLRSEDTAVYYCARVAPGNWGSPYFDYWGQGTLVTVSSASTKGPSVFPLAPSSKSTSGGTAALGCLVKDYFPEPVTVSWNSGALTSGVHTFPAVLQSSGLYSLSSVVTVPSSSLGTQTYICNVNHKPSNTKVDKKVEPKSCDKTHTCPPCPAPELLGGPSVFLFPPKPKDTLMISRTPEVTCVVVDVSHEDPEVKFNWYVDGVEVHNAKTKPREEQYNSTYRVVSVLTVLHQDWLNGKEYKCKVSNKALPAPIEKTISKAKGQPREPQVYTLPPSRDELTKNQVSLTCLVKGFYPSDIAVEWESNGQPENNYKTTPPVLDSDGSFFLYSKLTVDKSRWQQGNVFSCSVMHEALHNHYTQKSLSLSP

SEQ ID NO: 85 - protein, 214 aa, Artificial Sequence
  an artificially synthesized sequence
DIQMTQSPSSLSASVGDRVTITCRASQSIEDDLAWYQQKPGKAPKLLIYEASSLQSGVPSRFSGSGSGTDFTLTISSLQPEDFATYYCQQRDSSPLTFGQGTKVEIKRTVAAPSVFIFPPSDEQLKSGTASVVCLLNNFYPREAKVQWKVDNALQSGNSQESVTEQDSKDSTYSLSSTLTLSKADYEKHKVYACEVTHQGLSSPVTKSFNRGEC

SEQ ID NO: 86 - protein, 451 aa, Artificial Sequence
  an artificially synthesized sequence
QVQLVQSGAEVKKPGSSVKVSCKASGGTFSSYAISWVRQAPGQGLEWMGGIIPIFGTANYAQKFQGRVTITADESTSTAYMELSSLRSEDTAVYYCARPRWETAISSDAFDIWGQGTMVTVSSASTKGPSVFPLAPSSKSTSGGTAALGCLVKDYFPEPVTVSWNSGALTSGVHTFPAVLQSSGLYSLSSVVTVPSSSLGTQTYICNVNHKPSNTKVDKKVEPKSCDKTHTCPPCPAPELLGGPSVFLFPPKPKDTLMISRTPEVTCVVVDVSHEDPEVKFNWYVDGVEVHNAKTKPREEQYNSTYRVVSVLTVLHQDWLNGKEYKCKVSNKALPAPIEKTISKAKGQPREPQVYTLPPSRDELTKNQVSLTCLVKGFYPSDIAVEWESNGQPENNYKTTPPVLDSDGSFFLYSKLTVDKSRWQQGNVFSCSVMHEALHNHYTQKSLSLSP

SEQ ID NO: 87 - protein, 214 aa, Artificial Sequence
  an artificially synthesized sequence
DIQMTQSPSSLSASVGDRVTITCRASQSISDDLNWYQQKPGKAPKLLIYEASNLQSGVPSRFSGSGSGTDFTLTISSLQPEDFATYYCQQHSSSPLTFGQGTKVEIKRTVAAPSVFIFPPSDEQLKSGTASVVCLLNNFYPREAKVQWKVDNALQSGNSQESVTEQDSKDSTYSLSSTLTLSKADYEKHKVYACEVTHQGLSSPVTKSFNRGEC

SEQ ID NO: 88 - protein, 448 aa, Artificial Sequence
  an artificially synthesized sequence
QVQLVQSGAEVKKPGSSVKVSCKASGGTFSSYAISWVRQAPGQGLEWMGGIIPIFGTANYAQKFQGRVTITADESTSTAYMELSSLRSEDTAVYYCARGNGDYLEYFQHWGQGTLVTVSSASTKGPSVFPLAPSSKSTSGGTAALGCLVKDYFPEPVTVSWNSGALTSGVHTFPAVLQSSGLYSLSSVVTVPSSSLGTQTYICNVNHKPSNTKVDKKVEPKSCDKTHTCPPCPAPELLGGPSVFLFPPKPKDTLMISRTPEVTCVVVDVSHEDPEVKFNWYVDGVEVHNAKTKPREEQYNSTYRVVSVLTVLHQDWLNGKEYKCKVSNKALPAPIEKTISKAKGQPREPQVYTLPPSRDELTKNQVSLTCLVKGFYPSDIAVEWESNGQPENNYKTTPPVLDSDGSFFLYSKLTVDKSRWQQGNVFSCSVMHEALHNHYTQKSLSLSP

SEQ ID NO: 89 - protein, 214 aa, Artificial Sequence
  an artificially synthesized sequence
DIQMTQSPSSLSASVGDRVTITCRASQSISDDLAWYQQKPGKAPKLLIYEASNLQSGVPSRFSGSGSGTDFTLTISSLQPEDFATYYCQQRDSSPLTFGQGTKVEIKRTVAAPSVFIFPPSDEQLKSGTASVVCLLNNFYPREAKVQWKVDNALQSGNSQESVTEQDSKDSTYSLSSTLTLSKADYEKHKVYACEVTHQGLSSPVTKSFNRGEC

SEQ ID NO: 90 - protein, 452 aa, Artificial Sequence
  an artificially synthesized sequence
QVQLQQSGPGLVKPSETLSLTCTILGGSISGHYWSWIRQTPGKGLEWIGYIDYSGSTHYNPSLKSRVTMSVDTSKNQFSLKLSSVTAADTAMYYCARDNWDFGSGSYYNWFDPWGQGTLVTVSSASTKGPSVFPLAPSSKSTSGGTAALGCLVKDYFPEPVTVSWNSGALTSGVHTFPAVLQSSGLYSLSSVVTVPSSSLGTQTYICNVNHKPSNTKVDKKVEPKSCDKTHTCPPCPAPELLGGPSVFLFPPKPKDTLMISRTPEVTCVVVDVSHEDPEVKFNWYVDGVEVHNAKTKPREEQYNSTYRVVSVLTVLHQDWLNGKEYKCKVSNKALPAPIEKTISKAKGQPREPQVYTLPPSRDELTKNQVSLTCLVKGFYPSDIAVEWESNGQPENNYKTTPPVLDSDGSFFLYSKLTVDKSRWQQGNVFSCSVMHEALHNHYTQKSLSLSP

SEQ ID NO: 91 - protein, 214 aa, Artificial Sequence
  an artificially synthesized sequence
DIQMTQSPSSLSASVGDRVTITCRASQSIEDDLAWYQQKPGKAPKLLIYHASSLQSGVPSRFSGSGSGTDFTLTISSLQPEDFATYYCQQSDNSPLTFGQGTKVEIKRTVAAPSVFIFPPSDEQLKSGTASVVCLLNNFYPREAKVQWKVDNALQSGNSQESVTEQDSKDSTYSLSSTLTLSKADYEKHKVYACEVTHQGLSSPVTKSFNRGEC

SEQ ID NO: 92 - protein, 451 aa, Artificial Sequence
  an artificially synthesized sequence
QVQLVQSGAEVKKPGSSVKVSCKASGGTFSSYAISWVRQAPGQGLEWMGGIIPIFGTANYAQKFQGRVTITADESTSTAYMELSSLRSEDTAVYYCARPRWETAISSDAFDIWGQGTMVTVSSASTKGPSVFPLAPSSKSTSGGTAALGCLVKDYFPEPVTVSWNSGALTSGVHTFPAVLQSSGLYSLSSVVTVPSSSLGTQTYICNVNHKPSNTKVDKKVEPKSCDKTHTCPPCPAPELLGGPSVFLFPPKPKDTLMISRTPEVTCVVVDVSHEDPEVKFNWYVDGVEVHNAKTKPREEQYNSTYRVVSVLTVLHQDWLNGKEYKCKVSNKALPAPIEKTISKAKGQPREPQVYTLPPSRDELTKNQVSLTCLVKGFYPSDIAVEWESNGQPENNYKTTPPVLDSDGSFFLYSKLTVDKSRWQQGNVFSCSVMHEALHWHYTQKSLSLSP

SEQ ID NO: 93 - protein, 545 aa, Artificial Sequence
  an artificially synthesized sequence
QPPPPPPDATCHQVRSFFQRLQPGLKWVPETPVPGSDLQVCLPKGPTCCSRKMEEKYQLTARLNMEQLLQSASMELKFLIIQNAAVFQEAFEIVVRHAKNYTNAMFKNNYPSLTPQAFEFVGEFFTDVSLYILGSDINVDDMVNELFDSLFPVIYTQLMNPGLPDSALDINECLRGARRDLKVFGNFPKLIMTQVSKSLQVTRIFLQALNLGIEVINTTDHLKFSKDCGRMLTRMWYCSYCQGLMMVKPCGGYCNVVMQGCMAGVVEIDKYWREYILSLEELVNGMYRIYDMENVLLGLFSTIHDSIQYVQKNAGKLTTTIGKLCAHSQQRQYRSAYYPEDLFIDKKVLKVAHVEHEETLSSRRRELIQKLKSFISFYSALPGYICSHSPVAENDTLCWNGQELVERYSQKAARNGMKNQFNLHELKMKGPEPVVSQIIDKLKHINQLLRTMSMPKGRVLDKNLDEEGFEAGDCGDDEDECIGGAGDGMIKVKNQLRFLAELAYDLDVDDAPGNSQQATPKDNEISTFHNLGNVHSPLKHHHHHH

SEQ ID NO: 94 - protein, 443 aa, Artificial Sequence
  an artificially synthesized sequence
EVQLVETGGGVVQPGRSLRLSCAASGFTFSSYAMHWVRQAPGKGLEWVAVISYDGSNKYYADSVKGRFTISRDNSKNTLYLQMNSLRAEDTAVYYCARGAGMDVWGQGTTVTVSSASTKGPSVFPLAPSSKSTSGGTAALGCLVKDYFPEPVTVSWNSGALTSGVHTFPAVLQSSGLYSLSSVVTVPSSSLGTQTYICNVNHKPSNTKVDKKVEPKSCDKTHTCPPCPAPELLGGPSVFLFPPKPKDTLMISRTPEVTCVVVDVSHEDPEVKFNWYVDGVEVHNAKTKPREEQYNSTYRVVSVLTVLHQDWLNGKEYKCKVSNKALPAPIEKTISKAKGQPREPQVYTLPPSRDELTKNQVSLTCLVKGFYPSDIAVEWESNGQPENNYKTTPPVLDSDGSFFLYSKLTVDKSRWQQGNVFSCSVMHEALHNHYTQKSLSLSP

SEQ ID NO: 95 - protein, 214 aa, Artificial Sequence
  an artificially synthesized sequence
DIQMTQSPSSLSASVGDRVTITCRASQSIEDDLAWYQQKPGKAPKLLIYEASNLQSGVPSRFSGSGSGTDFTLTISSLQPEDFATYYCQQHDSYPLTFGQGTKVEIKRTVAAPSVFIFPPSDEQLKSGTASVVCLLNNFYPREAKVQWKVDNALQSGNSQESVTEQDSKDSTYSLSSTLTLSKADYEKHKVYACEVTHQGLSSPVTKSFNRGEC

SEQ ID NO: 96 - protein, 459 aa, Artificial Sequence
  an artificially synthesized sequence
QVQLVQSGGGVVQPGRSLRLSCAASGFTFSSYAMHWVRQAPGKGLEWVAVISYDGSNKYYADSVKGRFTISRDNSKNTLYLQMNSLRAEDTAVYYCAREPAGRHYYDSSGYYDYYYGMDVWGQGTMVTVSSASTKGPSVFPLAPSSKSTSGGTAALGCLVKDYFPEPVTVSWNSGALTSGVHTFPAVLQSSGLYSLSSVVTVPSSSLGTQTYICNVNHKPSNTKVDKKVEPKSCDKTHTCPPCPAPELLGGPSVFLFPPKPKDTLMISRTPEVTCVVVDVSHEDPEVKFNWYVDGVEVHNAKTKPREEQYNSTYRVVSVLTVLHQDWLNGKEYKCKVSNKALPAPIEKTISKAKGQPREPQVYTLPPSRDELTKNQVSLTCLVKGFYPSDIAVEWESNGQPENNYKTTPPVLDSDGSFFLYSKLTVDKSRWQQGNVFSCSVMHEALHNHYTQKSLSLSP

SEQ ID NO: 97 - protein, 214 aa, Artificial Sequence
  an artificially synthesized sequence
DIQMTQSPSSLSASVGDRVTITCRASQSISDDLNWYQQKPGKAPKLLIYEASNLQSGVPSRFSGSGSGTDFTLTISSLQPEDFATYYCQQYNSLPLTFGQGTKVEIKRTVAAPSVFIFPPSDEQLKSGTASVVCLLNNFYPREAKVQWKVDNALQSGNSQESVTEQDSKDSTYSLSSTLTLSKADYEKHKVYACEVTHQGLSSPVTKSFNRGEC

SEQ ID NO: 98 - protein, 451 aa, Artificial Sequence
  an artificially synthesized sequence
QVQLVETGGGLVQPGGSLRLSCAASGFTFSSYAMSWVRQAPGKGLEWVSAISGSGGSTYYADSVKGRFTISRDNSKNTLYLQMNSLRAEDTAVYYCAKDRTPYDFWSGYLDYWGQGTLVTVSSASTKGPSVFPLAPSSKSTSGGTAALGCLVKDYFPEPVTVSWNSGALTSGVHTFPAVLQSSGLYSLSSVVTVPSSSLGTQTYICNVNHKPSNTKVDKKVEPKSCDKTHTCPPCPAPELLGGPSVFLFPPKPKDTLMISRTPEVTCVVVDVSHEDPEVKFNWYVDGVEVHNAKTKPREEQYNSTYRVVSVLTVLHQDWLNGKEYKCKVSNKALPAPIEKTISKAKGQPREPQVYTLPPSRDELTKNQVSLTCLVKGFYPSDIAVEWESNGQPENNYKTTPPVLDSDGSFFLYSKLTVDKSRWQQGNVFSCSVMHEALHNHYTQKSLSLSP

SEQ ID NO: 99 - protein, 214 aa, Artificial Sequence
  an artificially synthesized sequence
DIQMTQSPSSLSASVGDRVTITCRASQSIEDDLAWYQQKPGKAPKLLIYEASNLQSGVPSRFSGSGSGTDFTLTISSLQPEDFATYYCQQRDSSPLTFGQGTKVEIKRTVAAPSVFIFPPSDEQLKSGTASVVCLLNNFYPREAKVQWKVDNALQSGNSQESVTEQDSKDSTYSLSSTLTLSKADYEKHKVYACEVTHQGLSSPVTKSFNRGEC

SEQ ID NO: 100 - protein, 451 aa, Artificial Sequence
  an artificially synthesized sequence
QVQLVQSGAEVKKPGASVKVSCKASGYTFTSYGISWVRQAPGQGLEWMGWISAYNGNTNYAQKLQGRVTMTTDTSTSTAYMELRSLRSDDTAVYYCARDSPLLWFGEPFFDYWGQGTLVTVSSASTKGPSVFPLAPSSKSTSGGTAALGCLVKDYFPEPVTVSWNSGALTSGVHTFPAVLQSSGLYSLSSVVTVPSSSLGTQTYICNVNHKPSNTKVDKKVEPKSCDKTHTCPPCPAPELLGGPSVFLFPPKPKDTLMISRTPEVTCVVVDVSHEDPEVKFNWYVDGVEVHNAKTKPREEQYNSTYRVVSVLTVLHQDWLNGKEYKCKVSNKALPAPIEKTISKAKGQPREPQVYTLPPSRDELTKNQVSLTCLVKGFYPSDIAVEWESNGQPENNYKTTPPVLDSDGSFFLYSKLTVDKSRWQQGNVFSCSVMHEALHNHYTQKSLSLSP

SEQ ID NO: 101 - protein, 214 aa, Artificial Sequence
  an artificially synthesized sequence
DIQMTQSPSSLSASVGDRVTITCRASQSIEDDLAWYQQKPGKAPKLLIYHASTLQSGVPSRFSGSGSGTDFTLTISSLQPEDFATYYCQQSDSYPLTFGQGTKVEIKRTVAAPSVFIFPPSDEQLKSGTASVVCLLNNFYPREAKVQWKVDNALQSGNSQESVTEQDSKDSTYSLSSTLTLSKADYEKHKVYACEVTHQGLSSPVTKSFNRGEC

SEQ ID NO: 102 - protein, 443 aa, Artificial Sequence
  an artificially synthesized sequence
QVQLVQSGAEVKKPGASVKVSCKASGYTFTDYEMHWVRQAPGQGLEWMGALDPKTGDTAYSQKFKGRVTLTADKSTSTAYMELSSLTSEDTAVYYCTRFYSYTYWGQGTLVTVSSASTKGPSVFPLAPSSKSTSGGTAALGCLVKDYFPEPVTVSWNSGALTSGVHTFPAVLQSSGLYSLSSVVTVPSSSLGTQTYICNVNHKPSNTKVDKKVEPKSCDKTHTCPPCPAPELLGGPSVFLFPPKPKDTLMISRTPEVTCVVVDVSHEDPEVKFNWYVDGVEVHNAKTKPREEQYNSTYRVVSVLTVLHQDWLNGKEYKCKVSNKALPAPIEKTISKAKGQPREPQVYTLPPSRDELTKNQVSLTCLVKGFYPSDIAVEWESNGQPENNYKTTPPVLDSDGSFFLYSKLTVDKSRWQQGNVFSCSVMHEALHNHYTQKSLSLSP

SEQ ID NO: 103 - protein, 219 aa, Artificial Sequence
  an artificially synthesized sequence
DVVMTQSPLSLPVTPGEPASISCRSSQSLVHSNRNTYLHWYLQKPGQSPQLLIYKVSNRFSGVPDRFSGSGSGTDFTLKISRVEAEDVGVYYCSQNTHVPPTFGQGTKLEIKRTVAAPSVFIFPPSDEQLKSGTASVVCLLNNFYPREAKVQWKVDNALQSGNSQESVTEQDSKDSTYSLSSTLTLSKADYEKHKVYACEVTHQGLSSPVTKSFNRGEC

SEQ ID NO: 104 - protein, 567 aa, Artificial Sequence
  an artificially synthesized sequence
QVQLQESGPGLVRPSQTLSLTCTVSGYSITSDHAWSWVRQPPGRGLEWIGYISYSGITTYNPSLKSRVTMLRDTSKNQFSLRLSSVTAADTAVYYCARSLARTTAMDYWGQGSLVTVSSASTQSPSVFPLTRCCKNIPSNATSVTLGCLATGYFPEPVMVTWDTGSLNGTTMTLPATTLTLSGHYATISLLTVSGAWAKQMFTCRVAHTPSSTDWVDNKTFSVCSRDFTPPTVKILQSSCDGGGHFPPTIQLLCLVSGYTPGTINITWLEDGQVMDVDLSTASTTQEGELASTQSELTLSQKHWLSDRTYTCQVTYQGHTFEDSTKKCADSNPRGVSAYLSRPSPFDLFIRKSPTITCLVVDLAPSKGTVNLTWSRASGKPVNHSTRKEEKQRNGTLTVTSTLPVGTRDWIEGETYQCRVTHPHLPRALMRSTTKTSGPRAAPEVYAFATPEWPGSRDKRTLACLIQNFMPEDISVQWLHNEVQLPDARHSTTQPRKTKGSGFFVFSRLEVTRAEWEQKDEFICRAVHEAASPSQTVQRAVSVNPGKGGGGSGLNDIFEAQKIEWHE

SEQ ID NO: 105 - protein, 438 aa, Artificial Sequence
  an artificially synthesized sequence
QSLEESGGDLVKPGGTLTLTCTASGYDFSSAYDMCWVRQAPGKGLEWIACIYTGDGVTYYASWAKGRFTISKTSSTTVTLQMTSLTAADTATYFCARGGDYYDLWGPGTLVTVSSGQPKAPSVFPLAPCCGDTPSSTVTLGCLVKGYLPEPVTVTWNSGTLTNGVRTFPSVRQSSGLYSLSSVVSVTSSSQPVTCNVAHPATNTKVDKTVAPSTCSKPMCPPPELLGGPSVFIFPPKPKDTLMISRTPEVTCVVVDVSQDDPEVQFTWYINNEQVRTARPPLREQQFNSTIRVVSTLPIAHQDWLRGKEFKCKVHNKALPAPIEKTISKARGQPLEPKVYTMGPPREELSSRSVSLTCMINGFYPSDISVEWEKNGKAEDNYKTTPTVLDSDGSYFLYSKLSVPTSEWQRGDVFTCSVMHEALHNHYTQKSISRSPGK

SEQ ID NO: 106 - protein, 215 aa, Artificial Sequence
  an artificially synthesized sequence
AIVMTQTPSSKSVPVGDTVTINCQASESVYSNYLAWFQQKPGQPPKRLIYGASTLDSGVSSRFKGSGSGTQFTLTINDVQCDDAATYYCAGYKSDNTDGIAFGGGTEVVVKGDPVAPTVLIFPPAADQVATGTVTIVCVANKYFPDVTVTWEVDGTTQTTGIENSKTPQNSADCTYNLSSTLTLTSTQYNSHKEYTCKVTQGTTSVVQSFNRGDC

SEQ ID NO: 107 - protein, 448 aa, Artificial Sequence
  an artificially synthesized sequence
QSVEESGGRLVTPGTPLTLTCTVSGFSLSSYDMSWVRQAPGKGLEWIGDIDTTTGTTIYATWAKGRFTISKTSTTVDLKITSPTTEDTATYFCARCAGGTGYCEDGLDPWGPGTLVTVSSASTKGPSVFPLAPSSKSTSGGTAALGCLVKDYFPEPVTVSWNSGALTSGVHTFPAVLQSSGLYSLSSVVTVPSSSLGTQTYICNVNHKPSNTKVDKKVEPKSCDKTHTCPPCPAPELLGGPSVFLFPPKPKDTLMISRTPEVTCVVVDVSHEDPEVKFNWYVDGVEVHNAKTKPREEQYNSTYRVVSVLTVLHQDWLNGKEYKCKVSNKALPAPIEKTISKAKGQPREPQVYTLPPSREEMTKNQVSLTCLVKGFYPSDIAVEWESNGQPENNYKTTPPVLDSDGSFFLYSKLTVDKSRWQQGNVFSCSVMHEALHNHYTQKSLSLSP

SEQ ID NO: 108 - protein, 217 aa, Artificial Sequence
  an artificially synthesized sequence
AFDMTQTPASVEVAVGGTVTINCQASQSIGSYLTWYQQKPGQPPKLLIYRASTLASGVSSRFKGSGSGTEFTLTISDLECADAATYYCQQDYSGSNVDNIFGGGTEVVVKRTVAAPSVFIFPPSDEQLKSGTASVVCLLNNFYPREAKVQWKVDNALQSGNSQESVTEQDSKDSTYSLSSTLTLSKADYEKHKVYACEVTHQGLSSPVTKSFNRGEC

SEQ ID NO: 109 - protein, 448 aa, Artificial Sequence
  an artificially synthesized sequence
QSVEESGGRLVTPGTPLTLTCTVSGFSLSSYDMSWVRQAPGKGLEWIGDIDTASGTTIYASWAKGRFTISKTSTTVDLKITSPTTEDTATYFCARCAGSSGYCENGLDPWGPGTLVTVSSASTKGPSVFPLAPSSKSTSGGTAALGCLVKDYFPEPVTVSWNSGALTSGVHTFPAVLQSSGLYSLSSVVTVPSSSLGTQTYICNVNHKPSNTKVDKKVEPKSCDKTHTCPPCPAPELLGGPSVFLFPPKPKDTLMISRTPEVTCVVVDVSHEDPEVKFNWYVDGVEVHNAKTKPREEQYNSTYRVVSVLTVLHQDWLNGKEYKCKVSNKALPAPIEKTISKAKGQPREPQVYTLPPSREEMTKNQVSLTCLVKGFYPSDIAVEWESNGQPENNYKTTPPVLDSDGSFFLYSKLTVDKSRWQQGNVFSCSVMHEALHNHYTQKSLSLSP

SEQ ID NO: 110 - protein, 217 aa, Artificial Sequence
  an artificially synthesized sequence
AIEMTQTPFSVSATVGGTVTINCQASQNINDYLSWYQQKPGQPPKLLIYKASTLASGVSSRFKGSGSGTEFTLTISDLECADAATYYCQQDYSGSDVDNIFGGGTEVVVKRTVAAPSVFIFPPSDEQLKSGTASVVCLLNNFYPREAKVQWKVDNALQSGNSQESVTEQDSKDSTYSLSSTLTLSKADYEKHKVYACEVTHQGLSSPVTKSFNRGEC

SEQ ID NO: 111 - protein, 449 aa, Artificial Sequence
  an artificially synthesized sequence
EVQLVESGGGLVQPGGSLRLSCAVSGYSITSGYSWNWIRQAPGKGLEWVASITYDGSTNYNPSVKGRITISRDDSKNTFYLQMNSLRAEDTAVYYCARGSHYFGHWHFAVWGQGTLVTVSSASTKGPSVFPLAPSSKSTSGGTAALGCLVKDYFPEPVTVSWNSGALTSGVHTFPAVLQSSGLYSLSSVVTVPSSSLGTQTYICNVNHKPSNTKVDKKVEPKSCDKTHTCPPCPAPELLGGPSVFLFPPKPKDTLMISRTPEVTCVVVDVSHEDPEVKFNWYVDGVEVHNAKTKPREEQYNSTYRVVSVLTVLHQDWLNGKEYKCKVSNKALPAPIEKTISKAKGQPREPQVYTLPPSRDELTKNQVSLTCLVKGFYPSDIAVEWESNGQPENNYKTTPPVLDSDGSFFLYSKLTVDKSRWQQGNVFSCSVMHEALHNHYTQKSLSLSP

SEQ ID NO: 112 - protein, 218 aa, Artificial Sequence
  an artificially synthesized sequence
DIQLTQSPSSLSASVGDRVTITCRASQSVDYDGDSYMNWYQQKPGKAPKLLIYAASYLESGVPSRFSGSGSGTDFTLTISSLQPEDFATYYCQQSHEDPYTFGQGTKVEIKRTVAAPSVFIFPPSDEQLKSGTASVVCLLNNFYPREAKVQWKVDNALQSGNSQESVTEQDSKDSTYSLSSTLTLSKADYEKHKVYACEVTHQGLSSPVTKSFNRGEC

SEQ ID NO: 113 - protein, 19 aa, Artificial sequence
  an artificially synthesized sequence
MGWSCIILFLVATATGVHS